European Patent Specification EP 4 133 097 B1, published April 29, 2026. Title: Improved methods of producing a lipidated protein. Applicant: Valneva Austria GmbH. The sequence listing filed with the application follows.

SEQUENCE LISTING (22 sequences)

SEQ ID NO: 1 - protein, 320 aa, Artificial Sequence
  Lip-S1D1-S2D1
  MISC_FEATURE (1)..(1): Lipidation
CSSFNEKGEVSEKIITRADGTRLEYTGIKSDGSGKAKEVLKNFTLEGKVANDKTTLVVKCGTVTLSKNISKSGEVSVELNDTDSSAATKKTAAWNSGTSTLTITVNSKKTKDLVFTKENTITVQQYDSNGTKLEGSAVEITKLDEICNALKGTSDKNNGSGSKEKNKDGKYSFNEKGELSAKTMTRENGTKLEYTEMKSDGTGKAKEVLKNFTLEGKVANDKVTLEVKCGTVTLSKEIAKSGEVTVALNDTNTTQATKKTGAWDSKTSTLTISVNSKKTTQLVFTKQDTITVQKYDSAGTNLEGTAVEIKTLDELCNALK

SEQ ID NO: 2 - protein, 322 aa, Artificial Sequence
  Lip-S4D1-S3hybD1
  MISC_FEATURE (1)..(1): Lipidation
CSSFNAKGELSEKTILRANGTRLEYTEIKSDGTGKAKEVLKDFALEGTLAADKTTLKVTCGTVVLSKHIPNSGEITVELNDSNSTQATKKTGKWDSNTSTLTISVNSKKTKNIVFTKEDTITVQKYDSAGTNLEGNAVEIKTLDELCNALKGTSDKNNGSGSKEKNKDGKYSFNEKGEVSEKILTRSNGTTLEYSQMTDAENATKAVETLKNGIKLPGNLVGGKTKLTVTCGTVTLSKNISKSGEITVALNDTETTPADKKTGEWKSDTSTLTISKNSQKTKQLVFTKENTITVQNYNRAGNALEGSPAEIKDLAELCAALK

SEQ ID NO: 3 - protein, 321 aa, Artificial Sequence
  Lip-S5D1-S6D1
  MISC_FEATURE (1)..(1): Lipidation
CSSFNEKGEISEKTIVRANGTRLEYTDIKSDKTGKAKEVLKDFTLEGTLAADGKTTLKVTCGTVTLSKNISKSGEITVALDDTDSSGNKKSGTWDSGTSTLTISKNRTKTKQLVFTKEDTITVQNYDSAGTNLEGKAVEITTLKELCNALKGTSDKNNGSGSKEKNKDGKYSFNGKGETSEKTIVRANGTRLEYTDIKSDGSGKAKEVLKDFTLEGTLAADGKTTLKVTCGTVVLSKNILKSGEITAALDDSDTTRATKKTGKWDSKTSTLTISVNSQKTKNLVFTKEDTITVQRYDSAGTNLEGKAVEITTLKELCNALK

SEQ ID NO: 4 - DNA, 1020 bp, Artificial Sequence
  Lip-S1D1-S2D1
atgaaagctactaaactggtactgggcgcggtaatcctgggttctactctgctggcaggttgctcaagcttcaacgaaaagggcgaagtcagcgaaaaaatcattacccgcgcagacggcacccgcctggaatacaccggcatcaaatcggacggcagcggcaaagcgaaagaagttctgaaaaactttaccctggaaggcaaagtcgcaaatgataaaaccaccctggtggtgaaatgcggcaccgttacgctgagcaaaaacattagtaaatccggtgaagtctctgtggaactgaatgataccgacagctctgcggccaccaagaaaaccgcagcttggaactcaggcacctcgacgctgaccattacggttaatagcaagaaaaccaaagatctggtcttcacgaaagaaaacaccatcacggtgcagcaatatgacagcaatggtaccaaactggaaggctccgctgtggaaatcacgaaactggatgaaatctgtaatgctctgaaaggtactagtgacaaaaacaatggctctggtagcaaagagaaaaacaaagatggcaagtactcattcaacgaaaaaggcgaactgtcggcgaaaacgatgacgcgtgaaaacggcaccaaactggaatatacggaaatgaaaagcgatggcaccggtaaagcgaaagaagttctgaaaaactttaccctggaaggcaaagtcgccaatgacaaagtcaccctggaagtgaaatgcggcaccgttacgctgtcaaaagaaattgcaaaatcgggtgaagtgaccgttgctctgaacgatacgaataccacgcaagcgaccaagaaaaccggcgcctgggacagcaaaacctctacgctgaccattagtgttaatagcaagaaaaccacgcagctggtcttcaccaaacaagatacgatcaccgtgcagaaatacgacagtgcgggtaccaacctggaaggcacggctgttgaaatcaaaaccctggacgaactgtgtaacgccctgaaa

SEQ ID NO: 5 - DNA, 1029 bp, Artificial Sequence
  Lip-S4D1-S3hybD1
atgaaagctactaaactggtactgggcgcggtaatcctgggttctactctgctggcaggttgctcaagcttcaatgctaagggcgaactgagcgaaaaaacgatcctgcgtgcgaatggcacccgtctggaatacaccgaaatcaaatccgatggtacgggcaaagcaaaggaagtcctgaaagattttgctctggaaggtaccctggcggccgacaaaaccacgctgaaggtgacgtgcggcaccgtggttctgagcaaacatattccgaactctggtgaaatcaccgttgaactgaacgatagcaattctacgcaggcaaccaaaaagacgggcaaatgggacagtaatacctccacgctgaccatttcagtcaactcgaaaaagaccaaaaatattgtgttcacgaaggaagatacgatcaccgttcaaaaatatgactccgcgggcaccaacctggaaggcaatgccgtcgaaatcaaaaccctggatgaactgtgtaacgccctgaagggtactagtgacaaaaacaatggctctggtagcaaagagaaaaacaaagatggcaagtactcattcaacgaaaaaggcgaagtgagcgaaaaaattctgacccgtagcaatggcaccaccctggaatatagccagatgaccgatgcagaaaatgcaaccaaagcagttgaaaccctgaaaaacggtattaaactgcctggtaatctggttggtggtaaaaccaaactgaccgttacctgtggcaccgttaccctgagcaaaaacattagcaaaagcggtgaaattaccgtggcactgaatgataccgaaaccacaccggcagacaaaaaaaccggtgaatggaaaagcgataccagcaccctgaccattagtaaaaatagccagaaaacaaaacagctggtgtttaccaaagaaaacaccattaccgtgcagaattataaccgtgcaggtaatgcactggaaggtagtccggcagaaattaaagatctggcagaactgtgtgcagccctgaaataa

SEQ ID NO: 6 - DNA, 1023 bp, Artificial Sequence
  Lip-S5D1-S6D1
atgaaagctactaaactggtactgggcgcggtaatcctgggttctactctgctggcaggttgctcaagcttcaacgaaaagggcgaaatctcagaaaaaaccatcgtccgcgctaacggcacccgcctggaatacaccgacatcaaatcagacaagaccggtaaagcgaaggaagttctgaaagattttacgctggaaggtaccctggcagcagacggtaaaaccacgctgaaggtgacctgcggtaccgttacgctgtccaaaaacattagtaagtccggcgaaatcacggtcgccctggatgacaccgatagctctggcaacaaaaagagcggtacctgggattcaggcacctcgacgctgaccatttctaaaaatcgtacgaaaaccaagcagctggtcttcacgaaagaagatacgatcaccgtgcaaaactatgacagcgcaggtaccaatctggaaggcaaagctgtggaaattaccacgctgaaagaactgtgtaatgctctgaaaggtactagtgacaaaaacaatggctctggtagcaaagagaaaaacaaagatggcaagtactcattcaacggcaaaggtgaaacgagcgaaaagaccatcgtgcgtgcgaacggtacccgcctggaatatacggacattaaatcggacggcagcggcaaagcaaaggaagtcctgaaagattttacgctggaaggtaccctggcagcagacggtaaaaccacgctgaaggtgacgtgcggcaccgtggttctgtcaaaaaacattctgaagtcgggtgaaatcaccgcagctctggatgacagcgataccacgcgtgctacgaaaaagaccggtaaatgggatagcaagacctctacgctgaccattagtgtcaactcccagaaaacgaagaatctggtgttcaccaaagaagatacgatcaccgttcaacgctatgacagtgcgggcaccaacctggaaggcaaagccgttgaaattaccacgctgaaagaactgtgtaatgctctgaaa

SEQ ID NO: 7 - protein, 958 aa, Artificial Sequence
  C-TAB.G5
MVTGVFKGPNGFEYFAPANTHNNNIEGQAIVYQNKFLTLNGKKYYFDNDSKAVTGWQTIDGKKYYFNLNTAEAATGWQTIDGKKYYFNLNTAEAATGWQTIDGKKYYFNTNTFIASTGYTSINGKHFYFNTDGIMQIGVFKGPNGFEYFAPANTHNNNIEGQAILYQNKFLTLNGKKYYFGSDSKAVTGLRTIDGKKYYFNTNTAVAVTGWQTINGKKYYFNTNTSIASTGYTIISGKHFYFNTDGIMQIGVFKGPDGFEYFAPANTDANNIEGQAIRYQNRFLYLHDNIYYFGNNSKAATGWVTIDGNRYYFEPNTAMGANGYKTIDNKNFYFRNGLPQIGVFKGSNGFEYFAPANTDANNIEGQAIRYQNRFLHLLGKIYYFGNNSKAVTGWQTINGKVYYFMPDTAMAAAGGLFEIDGVIYFFGVDGVKAPGIYGRSMHNLITGFVTVGDDKYYFNPINGGAASIGETIIDDKNYYFNQSGVLQTGVFSTEDGFKYFAPANTLDENLEGEAIDFTGKLIIDENIYYFDDNYRGAVEWKELDGEMHYFSPETGKAFKGLNQIGDYKYYFNSDGVMQKGFVSINDNKHYFDDSGVMKVGYTEIDGKHFYFAENGEMQIGVFNTEDGFKYFAHHNEDLGNEEGEEISYSGILNFNNKIYYFDDSFTAVVGWKDLEDGSKYYFDEDTAEAYIGLSLINDGQYYFNDDGIMQVGFVTINDKVFYFSDSGIIESGVQNIDDNYFYIDDNGIVQIGVFDTSDGYKYFAPANTVNDNIYGQAVEYSGLVRVGEDVYYFGETYTIETGWIYDMENESDKYYFNPETKKACKGINLIDDIKYYFDEKGIMRTGLISFENNNYYFNENGEMQFGYINIEDKMFYFGEDGVMQIGVFNTPDGFKYFAHQNTLDENFEGESINYTGWLDLDEKRYYFTDEYIAATGSVIIDGEEYYFDPDTAQLVISE

SEQ ID NO: 8 - protein, 957 aa, Artificial Sequence
  C-TAB.G5.1
VTGVFKGPNGFEYFAPANTHNNNIEGQAIVYQNKFLTLNGKKYYFDNDSKAVTGWQTIDGKKYYFNLNTAEAATGWQTIDGKKYYFNLNTAEAATGWQTIDGKKYYFNTNTFIASTGYTSINGKHFYFNTDGIMQIGVFKGPNGFEYFAPANTDANNIEGQAILYQNKFLTLNGKKYYFGSDSKAVTGLRTIDGKKYYFNTNTAVAVTGWQTINGKKYYFNTNTSIASTGYTIISGKHFYFNTDGIMQIGVFKGPDGFEYFAPANTDANNIEGQAIRYQNRFLYLHDNIYYFGNNSKAATGWVTIDGNRYYFEPNTAMGANGYKTIDNKNFYFRNGLPQIGVFKGSNGFEYFAPANTDANNIEGQAIRYQNRFLHLLGKIYYFGNNSKAVTGWQTINGKVYYFMPDTAMAAAGGLFEIDGVIYFFGVDGVKAPGIYGRSMHNLITGFVTVGDDKYYFNPINGGAASIGETIIDDKNYYFNQSGVLQTGVFSTEDGFKYFAPANTLDENLEGEAIDFTGKLIIDENIYYFDDNYRGAVEWKELDGEMHYFSPETGKAFKGLNQIGDYKYYFNSDGVMQKGFVSINDNKHYFDDSGVMKVGYTEIDGKHFYFAENGEMQIGVFNTEDGFKYFAHHNEDLGNEEGEEISYSGILNFNNKIYYFDDSFTAVVGWKDLEDGSKYYFDEDTAEAYIGLSLINDGQYYFNDDGIMQVGFVTINDKVFYFSDSGIIESGVQNIDDNYFYIDDNGIVQIGVFDTSDGYKYFAPANTVNDNIYGQAVEYSGLVRVGEDVYYFGETYTIETGWIYDMENESDKYYFNPETKKACKGINLIDDIKYYFDEKGIMRTGLISFENNNYYFNENGEMQFGYINIEDKMFYFGEDGVMQIGVFNTPDGFKYFAHQNTLDENFEGESINYTGWLDLDEKRYYFTDEYIAATGSVIIDGEEYYFDPDTAQLVISE

SEQ ID NO: 9 - DNA, 1557 bp, Artificial Sequence
  C-TAB.G5
atgcataatttgataactggatttgtgactgtaggcgatgataaatactactttaatccaattaatggtggagctgcttcaattggagagacaataattgatgacaaaaattattatttcaaccaaagtggagtgttacaaacaggtgtatttagtacagaagatggatttaaatattttgccccagctaatacacttgatgaaaacctagaaggagaagcaattgattttactggaaaattaattattgacgaaaatatttattattttgatgataattatagaggagctgtagaatggaaagaattagatggtgaaatgcactattttagcccagaaacaggtaaagcttttaaaggtctaaatcaaataggtgattataaatactatttcaattctgatggagttatgcaaaaaggatttgttagtataaatgataataaacactattttgatgattctggtgttatgaaagtaggttacactgaaatagatggcaagcatttctactttgctgaaaacggagaaatgcaaataggagtatttaatacagaagatggatttaaatattttgctcatcataatgaagatttaggaaatgaagaaggtgaagaaatctcatattctggtatattaaatttcaataataaaatttactattttgatgattcatttacagctgtagttggatggaaagatttagaggatggttcaaagtattattttgatgaagatacagcagaagcatatataggtttgtcattaataaatgatggtcaatattattttaatgatgatggaattatgcaagttggatttgtcactataaatgataaagtcttctacttctctgactctggaattatagaatctggagtacaaaacatagatgacaattatttctatatagatgataatggtatagttcaaattggtgtatttgatacttcagatggatataaatattttgcacctgctaatactgtaaatgataatatttacggacaagcagttgaatatagtggtttagttagagttggggaagatgtatattattttggagaaacatatacaattgagactggatggatatatgatatggaaaatgaaagtgataaatattatttcaatccagaaactaaaaaagcatgcaaaggtattaatttaattgatgatataaaatattattttgatgagaagggcataatgagaacgggtcttatatcatttgaaaataataattattactttaatgagaatggtgaaatgcaatttggttatataaatatagaagataagatgttctattttggtgaagatggtgtcatgcagattggagtatttaatacaccagatggatttaaatactttgcacatcaaaatactttggatgagaattttgagggagaatcaataaactatactggttggttagatttagatgaaaagagatattattttacagatgaatatattgcagcaactggttcagttattattgatggtgaggagtattattttgatcctgatacagctcaattagtgattagtgaatag

SEQ ID NO: 10 - DNA, 2885 bp, Artificial Sequence
  C-TAB.G5.1
ccatggttacaggtgttttcaaaggtccgaacggctttgaatattttgcaccggcaaatacccacaataataatattgaaggccaggccatcgtgtatcagaataaatttctgaccctgaacggcaaaaaatactatttcgataacgatagcaaagcagttaccggttggcaaaccattgatggcaaaaaatattacttcaacctgaataccgcagaagcagcaaccggctggcagacgatcgacggtaaaaagtactattttaacctgaacacagccgaagccgctacaggctggcagacaatagatgggaagaagtattattttaataccaatacctttattgccagcaccggctataccagcattaatggcaaacacttctattttaacaccgatggtattatgcagatcggtgtgtttaagggccctaatggttttgagtacttcgctccggctaataccgatgcaaataacatcgaaggtcaggcaattctgtaccagaacaaatttttaacgctgaacggtaagaaatattactttggtagcgattcaaaagccgttaccggtctgcgtacgatcgacggcaagaaatattatttcaatacaaacaccgcagttgccgtgacaggttggcagacgataaatggtaagaagtactacttcaacaccaataccagcattgcaagtaccggttataccattatcagcggcaaacacttttacttcaatacagacggcattatgcagattggcgttttcaaaggtccggatggtttcgagtactttgcccctgcaaatacagatgcaaacaatattgagggacaggcaattcgctatcagaatcgttttctgtatctgcacgataacatctattacttcggcaataattcaaaagcagccaccggttgggttacaattgatggtaatcgttattactttgagccgaataccgcaatgggtgcaaatggttataaaaccatcgataacaaaaatttttatttccgcaacggtctgccgcagattggtgtttttaagggtagcaatggcttcgagtattttgcgccagccaacaccgatgccaacaacattgaaggccaagcgattcgttatcaaaaccgctttctgcatctgctgggcaaaatttattactttggcaacaatagcaaagcggtgacgggctggcaaaccattaacggtaaagtttattatttcatgccggataccgctatggcagcagccggtggtctgtttgaaattgatggcgtgatttatttttttggcgtggatggtgttaaagcaccgggtatttatggtcgtagcatgcataatctgattaccggttttgttaccgtgggcgacgataaatactactttaatccgattaatggtggtgcagcaagcattggtgaaaccattatcgatgacaaaaactattattttaaccagagcggtgttctgcagacaggtgtttttagcaccgaagatggcttcaaatattttgctcctgcgaatacactggatgaaaatctggaaggtgaagcaattgattttaccggcaaactgatcatcgacgagaacatctactattttgatgataattatcgcggtgccgtggaatggaaagaactggatggtgaaatgcactattttagtccggaaaccggtaaagcctttaaaggtctgaatcagatcggcgattacaagtattactttaattcagatggcgtgatgcagaaaggctttgtgagcattaacgacaacaaacactattttgacgacagcggtgtgatgaaagtgggttataccgaaatcgacgggaaacatttttattttgccgaaaacggcgaaatgcagattggagtatttaataccgaggacggctttaaatactttgcccatcataatgaagatctgggtaatgaagaaggcgaagaaattagctatagcggcattctgaattttaataacaagatctattatttcgatgatagcttcaccgcagttgttggttggaaagatctggaagatggcagcaaatattattttgatgaagataccgcagaggcctatattggtctgagcctgattaatgatggccagtattatttcaacgatgatggtatcatgcaggttggttttgtgaccatcaacgataaagtgttctatttcagcgatagcggcattattgaaagcggtgttcagaacatcgacgataactatttctacatcgatgataacggtattgttcagattggcgtgtttgatacctccgatggttataaatatttcgcaccagccaataccgtgaacgataatatttatggtcaggcagttgaatattcaggtctggttcgtgttggcgaagatgtttattattttggcgaaacctataccattgaaaccggctggatctatgatatggaaaacgagagcgacaagtactatttcaatccggaaacgaaaaaagcctgcaaaggcattaatctgatcgacgatattaagtactactttgacgaaaaaggcattatgcgtaccggtctgattagctttgagaacaacaactattacttcaatgagaacggtgagatgcagtttggctatatcaacatcgaggacaaaatgttttattttggtgaggacggtgtgatgcagataggggtttttaatacaccggatgggtttaagtattttgcacatcagaacaccctggatgaaaactttgaaggcgaaagcattaattataccggttggctggatctggatgagaaacgttattatttcaccgacgaatacattgcagcaaccggtagcgttattattgatggtgaggaatattacttcgatccggatacagcacagctggttattagcgaataactcgag

SEQ ID NO: 11 - protein, 21 aa, Artificial Sequence
  Peptide linker
GTSDKNNGSGSKEKNKDGKYS

SEQ ID NO: 12 - protein, 961 aa, Artificial Sequence
  Lip-C-TAB.G5.1
  MISC_FEATURE (1)..(1): Lipidation
CSSFVTGVFKGPNGFEYFAPANTHNNNIEGQAIVYQNKFLTLNGKKYYFDNDSKAVTGWQTIDGKKYYFNLNTAEAATGWQTIDGKKYYFNLNTAEAATGWQTIDGKKYYFNTNTFIASTGYTSINGKHFYFNTDGIMQIGVFKGPNGFEYFAPANTDANNIEGQAILYQNKFLTLNGKKYYFGSDSKAVTGLRTIDGKKYYFNTNTAVAVTGWQTINGKKYYFNTNTSIASTGYTIISGKHFYFNTDGIMQIGVFKGPDGFEYFAPANTDANNIEGQAIRYQNRFLYLHDNIYYFGNNSKAATGWVTIDGNRYYFEPNTAMGANGYKTIDNKNFYFRNGLPQIGVFKGSNGFEYFAPANTDANNIEGQAIRYQNRFLHLLGKIYYFGNNSKAVTGWQTINGKVYYFMPDTAMAAAGGLFEIDGVIYFFGVDGVKAPGIYGRSMHNLITGFVTVGDDKYYFNPINGGAASIGETIIDDKNYYFNQSGVLQTGVFSTEDGFKYFAPANTLDENLEGEAIDFTGKLIIDENIYYFDDNYRGAVEWKELDGEMHYFSPETGKAFKGLNQIGDYKYYFNSDGVMQKGFVSINDNKHYFDDSGVMKVGYTEIDGKHFYFAENGEMQIGVFNTEDGFKYFAHHNEDLGNEEGEEISYSGILNFNNKIYYFDDSFTAVVGWKDLEDGSKYYFDEDTAEAYIGLSLINDGQYYFNDDGIMQVGFVTINDKVFYFSDSGIIESGVQNIDDNYFYIDDNGIVQIGVFDTSDGYKYFAPANTVNDNIYGQAVEYSGLVRVGEDVYYFGETYTIETGWIYDMENESDKYYFNPETKKACKGINLIDDIKYYFDEKGIMRTGLISFENNNYYFNENGEMQFGYINIEDKMFYFGEDGVMQIGVFNTPDGFKYFAHQNTLDENFEGESINYTGWLDLDEKRYYFTDEYIAATGSVIIDGEEYYFDPDTAQLVISE

SEQ ID NO: 13 - protein, 449 aa, Artificial Sequence
  Lip-ToxA-His
  MISC_FEATURE (1)..(1): Lipidation
CSSFVTGVFKGPNGFEYFAPANTHNNNIEGQAIVYQNKFLTLNGKKYYFDNDSKAVTGWQTIDGKKYYFNLNTAEAATGWQTIDGKKYYFNLNTAEAATGWQTIDGKKYYFNTNTFIASTGYTSINGKHFYFNTDGIMQIGVFKGPNGFEYFAPANTDANNIEGQAILYQNKFLTLNGKKYYFGSDSKAVTGLRTIDGKKYYFNTNTAVAVTGWQTINGKKYYFNTNTSIASTGYTIISGKHFYFNTDGIMQIGVFKGPDGFEYFAPANTDANNIEGQAIRYQNRFLYLHDNIYYFGNNSKAATGWVTIDGNRYYFEPNTAMGANGYKTIDNKNFYFRNGLPQIGVFKGSNGFEYFAPANTDANNIEGQAIRYQNRFLHLLGKIYYFGNNSKAVTGWQTINGKVYYFMPDTAMAAAGGLFEIDGVIYFFGVDGVKAPGIYGLEHHHHHH

SEQ ID NO: 14 - protein, 528 aa, Artificial Sequence
  Lip-ToxB-His
  MISC_FEATURE (1)..(1): Lipidation
CSSFNLITGFVTVGDDKYYFNPINGGAASIGETIIDDKNYYFNQSGVLQTGVFSTEDGFKYFAPANTLDENLEGEAIDFTGKLIIDENIYYFDDNYRGAVEWKELDGEMHYFSPETGKAFKGLNQIGDYKYYFNSDGVMQKGFVSINDNKHYFDDSGVMKVGYTEIDGKHFYFAENGEMQIGVFNTEDGFKYFAHHNEDLGNEEGEEISYSGILNFNNKIYYFDDSFTAVVGWKDLEDGSKYYFDEDTAEAYIGLSLINDGQYYFNDDGIMQVGFVTINDKVFYFSDSGIIESGVQNIDDNYFYIDDNGIVQIGVFDTSDGYKYFAPANTVNDNIYGQAVEYSGLVRVGEDVYYFGETYTIETGWIYDMENESDKYYFNPETKKACKGINLIDDIKYYFDEKGIMRTGLISFENNNYYFNENGEMQFGYINIEDKMFYFGEDGVMQIGVFNTPDGFKYFAHQNTLDENFEGESINYTGWLDLDEKRYYFTDEYIAATGSVIIDGEEYYFDPDTAQLVISELEHHHHHH

SEQ ID NO: 15 - protein, 1276 aa, Artificial Sequence
  LIP-Protein\S_2019-nCoV/Italy-INMI1
  MISC_FEATURE (1)..(1): Lipidation
CSSMFVFLVLLPLVSSQCVNLTTRTQLPPAYTNSFTRGVYYPDKVFRSSVLHSTQDLFLPFFSNVTWFHAIHVSGTNGTKRFDNPVLPFNDGVYFASTEKSNIIRGWIFGTTLDSKTQSLLIVNNATNVVIKVCEFQFCNDPFLGVYYHKNNKSWMESEFRVYSSANNCTFEYVSQPFLMDLEGKQGNFKNLREFVFKNIDGYFKIYSKHTPINLVRDLPQGFSALEPLVDLPIGINITRFQTLLALHRSYLTPGDSSSGWTAGAAAYYVGYLQPRTFLLKYNENGTITDAVDCALDPLSETKCTLKSFTVEKGIYQTSNFRVQPTESIVRFPNITNLCPFGEVFNATRFASVYAWNRKRISNCVADYSVLYNSASFSTFKCYGVSPTKLNDLCFTNVYADSFVIRGDEVRQIAPGQTGKIADYNYKLPDDFTGCVIAWNSNNLDSKVGGNYNYLYRLFRKSNLKPFERDISTEIYQAGSTPCNGVEGFNCYFPLQSYGFQPTNGVGYQPYRVVVLSFELLHAPATVCGPKKSTNLVKNKCVNFNFNGLTGTGVLTESNKKFLPFQQFGRDIADTTDAVRDPQTLEILDITPCSFGGVSVITPGTNTSNQVAVLYQDVNCTEVPVAIHADQLTPTWRVYSTGSNVFQTRAGCLIGAEHVNNSYECDIPIGAGICASYQTQTNSPRRARSVASQSIIAYTMSLGAENSVAYSNNSIAIPTNFTISVTTEILPVSMTKTSVDCTMYICGDSTECSNLLLQYGSFCTQLNRALTGIAVEQDKNTQEVFAQVKQIYKTPPIKDFGGFNFSQILPDPSKPSKRSFIEDLLFNKVTLADAGFIKQYGDCLGDIAARDLICAQKFNGLTVLPPLLTDEMIAQYTSALLAGTITSGWTFGAGAALQIPFAMQMAYRFNGIGVTQNVLYENQKLIANQFNSAIGKIQDSLSSTASALGKLQDVVNQNAQALNTLVKQLSSNFGAISSVLNDILSRLDKVEAEVQIDRLITGRLQSLQTYVTQQLIRAAEIRASANLAATKMSECVLGQSKRVDFCGKGYHLMSFPQSAPHGVVFLHVTYVPAQEKNFTTAPAICHDGKAHFPREGVFVSNGTHWFVTQRNFYEPQIITTDNTFVSGNCDVVIGIVNNTVYDPLQPELDSFKEELDKYFKNHTSPDVDLGDISGINASVVNIQKEIDRLNEVAKNLNESLIDLQELGKYEQYIKWPWYIWLGFIAGLIAIVMVTIMLCCMTSCCSCLKGCCSCGSCCKFDEDDSEPVLKGVKLHYT

SEQ ID NO: 16 - protein, 523 aa, Artificial Sequence
  L7F_A1_23 protein sequence
MSWKVVIIFSLLITPQHGLKESYLEESCSTITEGYLSVLRTGWYTNVFTLEVGDVENLTCADGPSLIKTELDLTKSALRELRTVSADQLAREEQIEQPRQSGCGAGATAGVAIAKTIRLESEVTAIKNALKKTNEAVSTLGNGVRVLATAVRELKDFVSKNLTRAINKNKCDIADLKMAVSFSQFNRRFLNVVRQFSDNAGITPAISLDLMTDAELARAVSNMPTSAGQIKLMLENRAMVRRKGFGFLIGVYGSSVIYMVQLPIFGVIDTPCWIVKAAPSCSEKKGNYACLLREDQGWYCQNAGSTVYYPNEKDCETRGDHVFCDTCAGINVAEQSKECNINISTTNYPCKVSTGRHPISMVALSPLGALVACYKGVSCSIGSNRVGIIKQLNKGCSYITNQDADTVTIDNTVYQLSKVEGEQHVIKGRPVSSSFDPVKFPEDQFNVALDQVFESIENSQALVDQSNRILSAGYIPEAPRDGQAYVRKDGEWVLLSTFLGGLVPRGSHHHHHHSAWSHPQFEK

SEQ ID NO: 17 - protein, 529 aa, Artificial Sequence
  sF_A1_K_L7 protein sequence
MSWKVVIIFSLLITPQHGLKESYLEESCSTITEGYLSVLRTGWYTNVFTLEVGDVENLTCADGPSLIKTELDLTKSALRELRTVSADQLAREEQIEQPRQSGCGAGATAGVAIAKTIRLESEVTAIKNALKKTNEAVSTLGNGVRVLAFAVRELKDFVSKNLTRALNKNKCDIADLKMAVSFSQFNRRFLNVVRQFSDNAGITPAISLDLMTDAELARAVSNMPTSAGQIKLMLENRAMVRRKGFGFLIGVYGSSVIYMVQLPIFGVIDTPCWIVKAAPSCSEKKGNYACLLREDQGWYCQNAGSTVYYPNEKDCETRGDHVFCDTCAGINVAEQSKECNINISTTNYPCKVSTGRHPISMVALSPLGALVACYKGVSCSIGSNRVGIIKQLNKGCSYITNQDADTVTIDNTVYQLSKVEGEQHVIKGRPVSSSFDPVKFPEDQFNVALDQVFESIENSQALVDQSNRILSSAESAIGGYIPEAPRDGQAYVRKDGEWVLLSTFLGGLVPRGSHHHHHHSAWSHPQFEK

SEQ ID NO: 18 - protein, 523 aa, Artificial Sequence
  L7F_A1_31 protein sequence
MSWKVVIIFSLLITPQHGLKESYLEESCSTITEGYLSVLRTGWYTNVFMLEVGDVENLTCADGPSLLKTELDLTKSALRNLRTVSADQLAREEQIEQPRQSGCGAGATAGVAIAKTIRLESEVTAIKNALKKTNEAVSTLGNGVRVLATMVRELKDFVSKNLTRAINKNKCDIADLKMAVSFSQFNRRFLNVVRQFSDNAGITPAISLDLMTDAELARAVSNMPTSAGQIKLMLENRAMVRRKGFGILIGVYGSSVIYMVQLPIFGVIDTPCWIVKAAPSCSEKKGNYACLLREDQGWYCQNAGSTVYYPNEKDCETRGDHVFCDTCAGINVAEQSKECNINISTTNYPCKVSTGRHPISMVALSPLGALVACYKGVSCSIGSNRVGIIKQLNKGCSYITNQDADTVTIDNTVYQLSKVEGEQHVIKGRPVSSSFDPVKFPEDQFNVALDQVFESIENSQALVDQSNRILSAGYIPEAPRDGQAYVRKDGEWVLLSTFLGGLVPRGSHHHHHHSAWSHPQFEK

SEQ ID NO: 19 - protein, 523 aa, Artificial Sequence
  L7F_A1_33 protein sequence
MSWKVVIIFSLLITPQHGLKESYLEESCSTITEGYLSVLRTGWYTNVFMLCVGDVENLTCADGPSLLKTELDLTKSALRELRTVSADQLAREEQIEQPRQSGCGAGATAGVAIAKTIRLESEVTAIKNALKKTNEAVSTLGNGVRVLATMVRELCDFVSKNLTRAINKNKCDIADLKMAVSFSQFNRRFLNVVRQFSDNAGITPAISLDLMTDAELARAVSNMPTSAGQIKLMLENRAMVRRKGFGFLIGVYGSDVIYMVQLPIFGVIDTPCWIVKAAPSCSEKKGNYACLLREDQGWYCQNAGSTVYYPNEKDCETRGDHVFCDTCAGINVAEQSKECNINISTTNYPCKVSTGRHPISMVALSPLGALVACYKGVSCSIGSNRVGIIKQLNKGCSYITNQDADTVTIDNTVYQLSKVEGEQHVIKGRPVSSSFDPVKFPEDQFNVALDQVFESIENSQALVDQSNRCCSAGYIPEAPRDGQAYVRKDGEWVLLSTFLGGLVPRGSHHHHHHSAWSHPQFEK

SEQ ID NO: 20 - protein, 529 aa, Artificial Sequence
  L7F_A1_4.2 protein sequence
MSWKVVIIFSLLITPQHGLKESYLEESCSTITEGYLSVLRTGWYTNVFMLEVGDVENLTCADGPSLIKTELDLTKSALRELRTVSADQLAREEQIEQPRQSGCGAGATAGVAIAKTIRLESEVTAWKNALKKTNEVVSTLGNGVRVLVTMVRELKDFVSKNLTRALNKNKCDIADLKMAVSFSQFNRRFLNVVRQFSDNAGITPAISLDLMTDAELARAVSNMPTSAGQIKLMLENRAMVRRKGFGFLIGVYGSSVIYMVQLPIFGVIDTPCWIVKAAPSCSEKKGNYACLLREDQGWYCQNAGSTVYYPNEKDCETRGDHVFCDTCAGINVAEQSKECNINISTTNYPCKVSTGRHPISMVALSPLGALVACYKGVSCSIGSNRVGIIKQLNKGCSYITNQDADTVTIDNTVYQLSKVEGEQHVIKGRPVSSSFDPVKFPEDQFNVALDQVFESIENSQALVDQSNRILSSAESAIGGYIPEAPRDGQAYVRKDGEWVLLSTFLGGLVPRGSHHHHHHSAWSHPQFEK

SEQ ID NO: 21 - protein, 540 aa, Artificial Sequence
  sF_A1_K-E294 protein sequence with substitutions  A113C, A339C, T160F, I177L and trimerization helper KLL
MSWKVVIIFSLLITPQHGLKESYLEESCSTITEGYLSVLRTGWYTNVFTLEVGDVENLTCADGPSLIKTELDLTKSALRELRTVSADQLAREEQIENPRQSRFVLGAIALGVCTAAAVTAGVAIAKTIRLESEVTAIKNALKKTNEAVSTLGNGVRVLAFAVRELKDFVSKNLTRALNKNKCDIADLKMAVSFSQFNRRFLNVVRQFSDNAGITPAISLDLMTDAELARAVSNMPTSAGQIKLMLENRAMVRRKGFGFLIGVYGSSVIYMVQLPIFGVIDTPCWIVKAAPSCSEKKGNYACLLREDQGWYCQNAGSTVYYPNEKDCETRGDHVFCDTACGINVAEQSKECNINISTTNYPCKVSTGRHPISMVALSPLGALVACYKGVSCSIGSNRVGIIKQLNKGCSYITNQDADTVTIDNTVYQLSKVEGEQHVIKGRPVSSSFDPVKFPEDQFNVALDQVFESIENSQALVDQSNRILSSAESAIGGYIPEAPRDGQAYVRKDGEWVLLSTFLGGLVPRGSHHHHHHSAWSHPQFEK

SEQ ID NO: 22 - protein, 538 aa, Artificial Sequence
  sF_A1_MFur protein sequence with deletion of amino acids at positions 103 to 111, replacement of R102 by a furin site KKRKRR and the substitution G294E, stabilized in post-fusion conformation
MSWKVVIIFSLLITPQHGLKESYLEESCSTITEGYLSVLRTGWYTNVFTLEVGDVENLTCADGPSLIKTELDLTKSALRELRTVSADQLAREEQIENPRQSKKRKRRVATAAAVTAGVAIAKTIRLESEVTAIKNALKKTNEAVSTLGNGVRVLATAVRELKDFVSKNLTRAINKNKCDIADLKMAVSFSQFNRRFLNVVRQFSDNAGITPAISLDLMTDAELARAVSNMPTSAGQIKLMLENRAMVRRKGFGFLIGVYGSSVIYMVQLPIFGVIDTPCWIVKAAPSCSEKKGNYACLLREDQGWYCQNAGSTVYYPNEKDCETRGDHVFCDTAAGINVAEQSKECNINISTTNYPCKVSTGRHPISMVALSPLGALVACYKGVSCSIGSNRVGIIKQLNKGCSYITNQDADTVTIDNTVYQLSKVEGEQHVIKGRPVSSSFDPVKFPEDQFNVALDQVFESIENSQALVDQSNRILSSAEKGNTSGRENLYFQGGGGSGYIPEAPRDGQAYVRKDGEWVLLSTFLGGIEGRHHHHHH